European Patent Application EP 4 674 862 A2, published January 7, 2026. Title: PEPTIDES FOR TREATMENT AND PREVENTION OFNONALCOHOLIC FATTY LIVER DISEASE AND FIBROSIS. Applicant: UNIVERSITE DE STRASBOURG. Application EP. The sequence listing filed with the application follows.

SEQUENCE LISTING (52 sequences)

SEQ ID NO: 1 - protein, 672 aa, Homo sapiens
MADVFPGNDSTASQDVANRFARKGALRQKNVHEVKDHKFIARFFKQPTFCSHCTDFIWGFGKQGFQCQVCCFVVHKRCHEFVTFSCPGADKGPDTDDPRSKHKFKIHTYGSPTFCDHCGSLLYGLIHQGMKCDTCDMNVHKQCVINVPSLCGMDHTEKRGRIYLKAEVADEKLHVTVRDAKNLIPMDPNGLSDPYVKLKLIPDPKNESKQKTKTIRSTLNPQWNESFTFKLKPSDKDRRLSVEIWDWDRTTRNDFMGSLSFGVSELMKMPASGWYKLLNQEEGEYYNVPIPEGDEEGNMELRQKFEKAKLGPAGNKVISPSEDRKQPSNNLDRVKLTDFNFLMVLGKGSFGKVMLADRKGTEELYAIKILKKDVVIQDDDVECTMVEKRVLALLDKPPFLTQLHSCFQTVDRLYFVMEYVNGGDLMYHIQQVGKFKEPQAVFYAAEISIGLFFLHKRGIIYRDLKLDNVMLDSEGHIKIADFGMCKEHMMDGVTTRTFCGTPDYIAPEIIAYQPYGKSVDWWAYGVLLYEMLAGQPPFDGEDEDELFQSIMEHNVSYPKSLSKEAVSVCKGLMTKHPAKRLGCGPEGERDVREHAFFRRIDWEKLENREIQPPFKPKVCGKGAENFDKFFTRGQPVLTPPDQLVIANIDQSDFEGFSYVNPQFVHPILQSAV

SEQ ID NO: 2 - protein, 257 aa, Homo sapiens
FNFLMVLGKGSFGKVMLADRKGTEELYAIKILKKDVVIQDDDVECTMVEKRVLALLDKPPFLTQLHSCFQTVDRLYFVMEYVNGGDLMYHIQQVGKFKEPQAVFYAAEISIGLFFLHKRGIIYRDLKLDNVMLDSEGHIKIADFGMCKEHMMDGVTTRTFCGTPDYIAPEIIAYQPYGKSVDWWAYGVLLYEMLAGQPPFDGEDEDELFQSIMEHNVSYPKSLSKEAVSVCKGLMTKHPAKRLGCGPEGERDVREHA

SEQ ID NO: 3 - protein, 12 aa, synthetic construct
  REGION 1..12: note = segment of kinase domain of alphaPKC
VECTMVEKRVLA

SEQ ID NO: 4 - protein, 8 aa, synthetic construct
  REGION 1..8: note = segment of kinase domain of alphaPKC
LMYHIQQV

SEQ ID NO: 5 - protein, 4 aa, synthetic construct
  REGION 1..4: note = segment of kinase domain of alphaPKC
PEII

SEQ ID NO: 6 - protein, 16 aa, synthetic construct
  REGION 1..16: note = segment of kinase domain of alphaPKC
SVDWWAYGVLLYEMLA

SEQ ID NO: 7 - protein, 12 aa, synthetic construct
  REGION 1..12: note = segment of kinase domain of alphaPKC
EDEDELFQSIME

SEQ ID NO: 8 - protein, 7 aa, synthetic construct
  REGION 1..7: note = segment of kinase domain of alphaPKC
GERDVRE

SEQ ID NO: 9 - protein, 12 aa, synthetic construct
  REGION 1..12: note = mutated segment of kinase domain of alphaPKC
  SITE 5: note = X is any amino acid except R, M and P
VECTXVEKRVLA

SEQ ID NO: 10 - protein, 12 aa, synthetic construct
  REGION 1..12: note = mutated segment of kinase domain of alphaPKC
  SITE 9: note = X is any amino acid except M, P and R
VECTMVEKXVLA

SEQ ID NO: 11 - protein, 12 aa, synthetic construct
  REGION 1..12: note = mutated segment of kinase domain of alphaPKC
  SITE 5: note = X is any amino acid except M, P and R
  SITE 9: note = X is any amino acid except M, P and R
VECTXVEKXVLA

SEQ ID NO: 12 - protein, 8 aa, synthetic construct
  REGION 1..8: note = mutated segment of kinase domain of alphaPKC
  SITE 2: note = X is any amino acid except M, P and R
LXYHIQQV

SEQ ID NO: 13 - protein, 16 aa, synthetic construct
  REGION 1..16: note = mutated segment of kinase domain of alphaPKC
  SITE 14: note = X is any amino acid except M, P and R
SVDWWAYGVLLYEXLA

SEQ ID NO: 14 - protein, 12 aa, synthetic construct
  REGION 1..12: note = mutated segment of kinase domain of alphaPKC
  SITE 11: note = X is any amino acid except M, P and R
EDEDELFQSIXE

SEQ ID NO: 15 - protein, 7 aa, synthetic construct
  REGION 1..7: note = mutated segment of kinase domain of alphaPKC
  SITE 3: note = X is any amino acid except M, P and R
GEXDVRE

SEQ ID NO: 16 - protein, 7 aa, synthetic construct
  REGION 1..7: note = mutated segment of kinase domain of alphaPKC
  SITE 6: note = X is any amino acid except M, P and R
GERDVXE

SEQ ID NO: 17 - protein, 7 aa, synthetic construct
  REGION 1..7: note = mutated segment of kinase domain of alphaPKC
  SITE 3: note = X is any amino acid except M, P and R
  SITE 6: note = X is any amino acid except M, P and R
GEXDVXE

SEQ ID NO: 18 - skipped

SEQ ID NO: 19 - protein, 12 aa, synthetic construct
  REGION 1..12: note = mutated segment of kinase domain of alphaPKC
VECTTVEKEVLA

SEQ ID NO: 20 - protein, 25 aa, synthetic construct
  REGION 1..25: note = mutated segment of kinase domain of alphaPKC
  SITE 5: note = X is any amino acid except M, P and R
  SITE 9: note = X is any amino acid except M, P and R
  REGION 17..18: note = X is any amino acid except M, P and R
VECTXVEKXVLALLDKXXFLTQLHS

SEQ ID NO: 21 - protein, 25 aa, synthetic construct
  REGION 1..25: note = mutated segment of kinase domain of alphaPKC
  REGION 17..18: note = X is any amino acid except M, P and R
VECTMVEKRVLALLDKXXFLTQLHS

SEQ ID NO: 22 - protein, 25 aa, synthetic construct
  REGION 1..25: note = mutated segment of kinase domain of alphaPKC
  SITE 5: note = X is any amino acid except M, P and R
VECTXVEKRVLALLDKPPFLTQLHS

SEQ ID NO: 23 - protein, 25 aa, synthetic construct
  REGION 1..25: note = mutated segment of kinase domain of alphaPKC
  SITE 9: note = X is any amino acid except M, P and R
VECTMVEKXVLALLDKPPFLTQLHS

SEQ ID NO: 24 - protein, 13 aa, synthetic construct
  REGION 1..13: note = mutated segment of kinase domain of alphaPKC
  SITE 6: note = X is any amino acid derivative suitable for stapling
  SITE 13: note = X is any amino acid derivative suitable for stapling
VECTMXEKRVLAX

SEQ ID NO: 25 - protein, 13 aa, synthetic construct
  REGION 1..13: note = mutated segment of kinase domain of alphaPKC
  SITE 5: note = X is any amino acid except M, P and R
  SITE 6: note = X is any amino acid derivative suitable for stapling
  SITE 13: note = X is any amino acid derivative suitable for stapling
VECTXXEKRVLAX

SEQ ID NO: 26 - protein, 13 aa, synthetic construct
  REGION 1..13: note = mutated segment of kinase domain of alphaPKC
  SITE 6: note = X is any amino acid derivative suitable for stapling
  SITE 9: note = X is any amino acid except M, P and R
  SITE 13: note = X is any amino acid derivative suitable for stapling
VECTMXEKXVLAX

SEQ ID NO: 27 - protein, 13 aa, synthetic construct
  REGION 1..13: note = mutated segment of kinase domain of alphaPKC
  SITE 5: note = X is any amino acid except M, P and R
  SITE 6: note = X is any amino acid derivative suitable for stapling
  SITE 9: note = X is any amino acid except M, P and R
  SITE 13: note = X is any amino acid derivative suitable for stapling
VECTXXEKXVLAX

SEQ ID NO: 28 - protein, 25 aa, synthetic construct
  REGION 1..25: note = mutated segment of kinase domain of alphaPKC
  SITE 5: note = X is any amino acid except M, P and R
  SITE 6: note = X is any amino acid derivative suitable for stapling
  SITE 9: note = X is any amino acid except M, P and R
  SITE 13: note = X is any amino acid derivative suitable for stapling
  REGION 17..18: note = X is any amino acid except M, P and R
VECTXXEKXVLAXLDKXXFLTQLHS

SEQ ID NO: 29 - protein, 25 aa, synthetic construct
  REGION 1..25: note = mutated segment of kinase domain of alphaPKC
  SITE 6: note = X is any amino acid derivative suitable for stapling
  SITE 13: note = X is any amino acid derivative suitable for stapling
  REGION 17..18: note = X is any amino acid except M, P and R
VECTMXEKRVLAXLDKXXFLTQLHS

SEQ ID NO: 30 - protein, 25 aa, synthetic construct
  REGION 1..25: note = mutated segment of kinase domain of alphaPKC
  SITE 5: note = X is any amino acid except M, P and R
  SITE 6: note = X is any amino acid derivative suitable for stapling
  SITE 13: note = X is any amino acid derivative suitable for stapling
VECTXXEKRVLAXLDKPPFLTQLHS

SEQ ID NO: 31 - protein, 25 aa, synthetic construct
  REGION 1..25: note = mutated segment of kinase domain of alphaPKC
  SITE 6: note = X is any amino acid derivative suitable for stapling
  SITE 9: note = X is any amino acid except M, P and R
  SITE 13: note = X is any amino acid derivative suitable for stapling
VECTMXEKXVLAXLDKPPFLTQLHS

SEQ ID NO: 32 - protein, 25 aa, synthetic construct
  REGION 1..25: note = mutated segment of kinase domain of alphaPKC
VECTTREKEVLASLDKAAFLTQLHS

SEQ ID NO: 33 - protein, 8 aa, synthetic construct
  REGION 1..8: note = protein transduction domain
RRRRRRRR

SEQ ID NO: 34 - protein, 15 aa, synthetic construct
  REGION 1..15: note = protein transduction domain
RRPRRPRRPRRPRRP

SEQ ID NO: 35 - protein, 16 aa, synthetic construct
  REGION 1..16: note = penetratin peptide
RQIKIWFQNRRMKWKK

SEQ ID NO: 36 - protein, 11 aa, synthetic construct
  REGION 1..11: note = HIV-tat
YGRKKRRQRRR

SEQ ID NO: 37 - DNA, 20 bp, synthetic construct
  misc_feature 1..20: note = primer
  source 1..20: mol_type = other DNA
tgctttggtttctgggactt

SEQ ID NO: 38 - DNA, 20 bp, synthetic construct
  misc_feature 1..20: note = primer
  source 1..20: mol_type = other DNA
gctctagccgaacacgaatc

SEQ ID NO: 39 - DNA, 22 bp, synthetic construct
  misc_feature 1..22: note = primer
  source 1..22: mol_type = other DNA
tggacaaagtagacggagtgtc

SEQ ID NO: 40 - DNA, 20 bp, synthetic construct
  misc_feature 1..20: note = primer
  source 1..20: mol_type = other DNA
tagcaaggcctgtcccatac

SEQ ID NO: 41 - DNA, 20 bp, synthetic construct
  misc_feature 1..20: note = primer
  source 1..20: mol_type = other DNA
tgagaacttgccaccgtatg

SEQ ID NO: 42 - DNA, 20 bp, synthetic construct
  misc_feature 1..20: note = primer
  source 1..20: mol_type = other DNA
ggcaggtaggcccctatatc

SEQ ID NO: 43 - DNA, 20 bp, synthetic construct
  misc_feature 1..20: note = primer
  source 1..20: mol_type = other DNA
gtttcatccgggtcttcatc

SEQ ID NO: 44 - DNA, 20 bp, synthetic construct
  misc_feature 1..20: note = primer
  source 1..20: mol_type = other DNA
gtgtctgtgccctcgaaaat

SEQ ID NO: 45 - DNA, 20 bp, synthetic construct
  misc_feature 1..20: note = primer
  source 1..20: mol_type = other DNA
aagttctctgcctcccgatt

SEQ ID NO: 46 - DNA, 20 bp, synthetic construct
  misc_feature 1..20: note = primer
  source 1..20: mol_type = other DNA
caaagcgttgctggaagttt

SEQ ID NO: 47 - DNA, 20 bp, synthetic construct
  misc_feature 1..20: note = primer
  source 1..20: mol_type = other DNA
tcgattccctcctacactgc

SEQ ID NO: 48 - DNA, 20 bp, synthetic construct
  misc_feature 1..20: note = primer
  source 1..20: mol_type = other DNA
ttggtggtactggctcatca

SEQ ID NO: 49 - protein, 25 aa, synthetic construct
  REGION 1..25: note = Stapled peptide sequence A
  SITE 6: note = X is any amino acid derivative suitable for stapling
  SITE 13: note = X is any amino acid derivative suitable for stapling
VECTMXEKRVLAXLDKPPFLTQLHS

SEQ ID NO: 50 - protein, 21 aa, synthetic construct
  REGION 1..21: note = Stapled peptide sequence B
  SITE 2: note = X is any amino acid derivative suitable for stapling
  SITE 9: note = X is any amino acid derivative suitable for stapling
SXCKGLMTXHPAKRLGCGPEG

SEQ ID NO: 51 - protein, 26 aa, synthetic construct
  REGION 1..26: note = Scrambled peptide sequence A
KEVPVDTCHLTLMLLFRSVALKQHPE

SEQ ID NO: 52 - protein, 21 aa, synthetic construct
  REGION 1..21: note = Scrambled peptide sequence B
SAECKGRHGTPPGKLMICKGL